European Patent Specification EP 4 053 272 B1, published October 1, 2025. Title: NOVEL SERINE PROTEASE VARIANT. Applicant: CJ CheilJedang Corporation. The sequence listing filed with the application follows.

SEQUENCE LISTING (48 sequences)

SEQ ID NO: 1 - DNA, 6922 bp, Artificial Sequence
  pBE-S-TFP
actagtgttcttttctgtatgaaaatagttatttcgagtctctacggaaatagcgagagatgatatacctaaatagagataaaatcatctcaaaaaaatgggtctactaaaatattattccatctattacaataaattcacagaatagtcttttaagtaagtctactctgaacttaagcaaaaggagagggacgcgtgtgagaagcaaaaaattgtggatcagcttgttgtttgcgttaacgttaatctttacgatggcgttcagcaacatgtctgcgcaggctgcggccggtgcacatatgcaagagctggcgttgaaacgggacctcggcctctctgacgcagaagtagccgaactccgggctgctgaggcggaagcggtcgagctcgaggaggagctccgcgattcattagggtcagacttcggcggtgtatatctggatgctgacaccaccgaaattacggtcgcggtaaccgacccggcagcggtaagtcgtgtcgacgcggatgatgtcacagttgatgttgtcgatttcggggaaacagctttgaatgattttgtggcttcattaaatgccattgccgacacggcagaccctaaagtcactggatggtataccgatctcgaaagtgatgccgtagtcattacgaccttgcgtggcgggactcctgctgccgaggaacttgctgagagagcgggtctcgacgaaagagccgttcggattgtggaagaagatgaagaaccacagagcttggctgcaattattggtggaaacccgtactatttcggaaattacagatgcagtatcgggtttagtgtccgtcagggctctcaaacgggattcgcgaccgcaggccactgcggatccacggggacgcgtgtgtcttctccttcaggaacagttgcaggaagttatttcccgggtcgcgatatgggctgggtgcggattacatcagcagatactgtaacaccactcgtaaatcggtataatgggggaactgttacggtcactgggtcacaagaagctgccaccggatcctccgtttgtcgctctggagcaacaacgggctggcgctgcggaactatccaatcaaaaaaccaaacggttcgctatgcagaagggactgttactggtttaacaagaactacagcctgtgctgaaggtggggattctggagggccatggctcacaggtagccaggcgcaaggggttacaagcggcggaacaggcgattgcagaagtggagggattacctttttccaaccaatcaatccattgcttagctatttcggccttcaattagtgaccggctgaaagcttgtcgacctgcagtctagacatcaccatcatcaccactaatgcggtagtttatcacagttaaattgctaacgcagtcaggcaccgtgtatgaaatctaacaatgcgctcatcgtcatcctcggcaccgtcaccctggatgctgtaggcataggcttggttatgccggtactgccgggcctatttcactttttgcattctacaaactgcataactattatgtaaatcgctcctttttaggtggcacaaatgtgaggcattttcgctctttccggcaaccacttccaagtaaagtataacacactatactttatattcataaagtgtgtgctctgcgaggctgtcggcagtgccgaccaaaaccataaaacctttaagacctttcttttttttacgagaaaaaagaaacaaaaaaacctgccctctgccacctcagcaaaggggggttttgctctcgtgctcgtttaaaaatcagcaagggacaggtagtattttttgagaagatcactcaaaaaatctccacctttaaacccttgccaatttttattttgtccgttttgtctagcttaccgaaagccagactcagcaagaataaaatttttattgtctttcggttttctagtgtaacggacaaaaccactcaaaataaaaaagatacaagagaggtctctcgtatcttttattcagcaatcgcgcccgattgctgaacagattaataatagattttagctttttatttgttgaaaaaagctaatcaaattgttgtcgggatcaattactgcaaagtctcgttcatcccaccactgatcttttaatgatgtattggggtgcaaaatgcccaaaggcttaatatgttgatataattcatcaattccctctacttcaatgcggcaactagcagtaccagcaataaacgactccgcacctgtacaaaccggtgaatcattactacgagagcgccagccttcatcacttgcctcccatagatgaatccgaacctcattacacattagaactgcgaatccatcttcatggtgaaccaaagtgaaacctagtttatcgcaataaaaacctatactctttttaatatccccgactggcaatgccgggatagactgtaacattctcacgcataaaatcccctttcattttctaatgtaaatctattaccttattattaattcaattcgctcataattaatcctttttcttattacgcaaaatggcccgatttaagcacaccctttattccgttaatgcgccatgacagccatgataattactaatactaggagaagttaataaatacgagcaaaaggccagcaaaaggccaggaaccgtaaaaaggccgcgttgctggcgtttttccataggctccgcccccctgacgagcatcacaaaaatcgacgctcaagtcagaggtggcgaaacccgacaggactataaagataccaggcgtttccccctggaagctccctcgtgcgctctcctgttccgaccctgccgcttaccggatacctgtccgcctttctcccttcgggaagcgtggcgctttctcatagctcacgctgtaggtatctcagttcggtgtaggtcgttcgctccaagctgggctgtgtgcacgaaccccccgttcagcccgaccgctgcgccttatccggtaactatcgtcttgagtccaacccggtaagacacgacttatcgccactggcagcagccactggtaacaggattagcagagcgaggtatgtaggcggtgctacagagttcttgaagtggtggcctaactacggctacactagaagaacagtatttggtatctgcgctctgctgaagccagttaccttcggaaaaagagttggtagctcttgatccggcaaacaaaccaccgctggtagcggtggtttttttgtttgcaagcagcagattacgcgcagaaaaaaaggatctcaagaagatcctttgatcttttctacggggtctgacgctcagtggaacgaaaactcacgttaagggattttggtcatgagattatcaaaaaggatcttcacctagatccttttaaattaaaaatgaagttttaaatcaatctaaagtatatatgagtaaacttggtctgacagttaccaatgcttaatcagtgaggcacctatctcagcgatctgtctatttcgttcatccatagttgcctgactccccgtcgtgtagataactacgatacgggagggcttaccatctggccccagtgctgcaatgataccgcgagacccacgctcaccggctccagatttatcagcaataaaccagccagccggaagggccgagcgcagaagtggtcctgcaactttatccgcctccatccagtctattaattgttgccgggaagctagagtaagtagttcgccagttaatagtttgcgcaacgttgttgccattgctacaggcatcgtggtgtcacgctcgtcgtttggtatggcttcattcagctccggttcccaacgatcaaggcgagttacatgatcccccatgttgtgcaaaaaagcggttagctccttcggtcctccgatcgttgtcagaagtaagttggccgcagtgttatcactcatggttatggcagcactgcataattctcttactgtcatgccatccgtaagatgcttttctgtgactggtgagtactcaaccaagtcattctgagaatagtgtatgcggcgaccgagttgctcttgcccggcgtcaatacgggataataccgcgccacatagcagaactttaaaagtgctcatcattggaaaacgttcttcggggcgaaaactctcaaggatcttaccgctgttgagatccagttcgatgtaacccactcgtgcacccaactgatcttcagcatcttttactttcaccagcgtttctgggtgagcaaaaacaggaaggcaaaatgccgcaaaaaagggaataagggcgacacggaaatgttgaatactcatactcttcctttttcaatattattgaagcatttatcagggttattgtctcatgagcggatacatatttgaatgtatttagaaaaataaacaaataggggttccgcgcacatttccccgaaaagtgccacctgacgtctaagaaaccattattatcatgacattaacctataaaaataggcgtatcacgaggccctttcgtctcgcgcgtttcggtgatgacggtgaaaacctctgacagtaaccaacatgattaacaattattagaggtcatcgttcaaaatggtatgcgttttgacacatccactatatatccgtgtcgttctgtccactcctgaatcccattccagaaattctctagcgattccagaagtttctcagagtcggaaagttgaccagacattacgaactggcacagatggtcataacctgaaggaagatctgattgcttaactgcttcagttaagaccgaagcgctcgtcgtataacagatgcgatgatgcagaccaatcaacatggcacctgccattgctacctgtacagtcaaggatggtagaaatgttgtcggtccttgcacacgaatattacgccatttgcctgcatattcaaacagctcttctacgataagggcacaaatcgcatcgtggaacgtttgggcttctaccgatttagcagtttgatacactttctctaagtatccacctgaatcataaatcggcaaaatagagaaaaattgaccatgtgtaagcggccaatctgattccacctgagatgcataatctagtagaatctcttcgctatcaaaattcacttccaccttccactcaccggttgtccattcatggctgaactctgcttcctctgttgacatgacacacatcatctcaatatccgaatagggcccatcagtctgacgaccaagagagccataaacaccaatagccttaacatcatccccatatttatccaatattcgttccttaatttcatgaacaatcttcattctttcttctctagtcattattattggtccattcactattctcattcccttttcagataattttagatttgcttttctaaataagaatatttggagagcaccgttcttattcagctattaataactcgtcttcctaagcatccttcaatccttttaataacaattatagcatctaatcttcaacaaactggcccgtttgttgaactactctttaataaaataatttttccgttcccaattccacattgcaataatagaaaatccatcttcatcggctttttcgtcatcatctgtatgaatcaaatcgccttcttctgtgtcatcaaggtttaattttttatgtatttcttttaacaaaccaccataggagattaaccttttacggtgtaaaccttcctccaaatcagacaaacgtttcaaattcttttcttcatcatcggtcataaaatccgtatcctttacaggatattttgcagtttcgtcaattgccgattgtatatccgatttatatttatttttcggtcgaatcatttgaacttttacatttggatcatagtctaatttcattgcctttttccaaaattgaatccattgtttttgattcacgtagttttctgtattcttaaaataagttggttccacacataccaatacatgcatgtgctgattataagaattatctttattatttattgtcacttccgttgcacgcataaaaccaacaagatttttattaatttttttatattgcatcattcggcgaaatccttgagccatatctgacaaactcttatttaattcttcgccatcataaacatttttaactgttaatgtgagaaacaaccaacgaactgttggcttttgtttaataacttcagcaacaaccttttgtgactgaatgccatgtttcattgctctcctccagttgcacattggacaaagcctggatttacaaaaccacactcgatacaactttctttcgcctgtttcacgattttgtttatactctaatatttcagcacaatcttttactctttcagcctttttaaattcaagaatatgcagaagttcaaagtaatcaacattagcgattttcttttctctccatggtctcacttttccactttttgtcttgtccactaaaacccttgatttttcatctgaataaatgctactattaggacacataatattaaaagaaacccccatctatttagttatttgtttagtcacttataactttaacagatggggtttttctgtgcaaccaattttaagggttttcaatactttaaaacacatacataccaacacttcaacgcacctttcagcaactaaaataaaaatgacgttatttctatatgtatcaagataagaaagaacaagttcaaaaccatcaaaaaaagacaccttttcaggtgctttttttattttataaactcattccctgatctcgacttcgttctttttttacctctcggttatgagttagttcaaattcgttctttttaggttctaaatcgtgtttttcttggaattgtgctgttttatcctttaccttgtctacaaaccccttaaaaacgtttttaaaggcttttaagccgtctgtacgttcctaa

SEQ ID NO: 2 - protein, 338 aa, Unknown
  Thermobifida fusca
MQELALKRDLGLSDAEVAELRAAEAEAVELEEELRDSLGSDFGGVYLDADTTEITVAVTDPAAVSRVDADDVTVDVVDFGETALNDFVASLNAIADTADPKVTGWYTDLESDAVVITTLRGGTPAAEELAERAGLDERAVRIVEEDEEPQSLAAIIGGNPYYFGNYRCSIGFSVRQGSQTGFATAGHCGSTGTRVSSPSGTVAGSYFPGRDMGWVRITSADTVTPLVNRYNGGTVTVTGSQEAATGSSVCRSGATTGWRCGTIQSKNQTVRYAEGTVTGLTRTTACAEGGDSGGPWLTGSQAQGVTSGGTGDCRSGGITFFQPINPLLSYFGLQLVTG

SEQ ID NO: 3 - protein, 338 aa, Artificial Sequence
  Thermobifida fusca (F163Y)
MQELALKRDLGLSDAEVAELRAAEAEAVELEEELRDSLGSDFGGVYLDADTTEITVAVTDPAAVSRVDADDVTVDVVDFGETALNDFVASLNAIADTADPKVTGWYTDLESDAVVITTLRGGTPAAEELAERAGLDERAVRIVEEDEEPQSLAAIIGGNPYYYGNYRCSIGFSVRQGSQTGFATAGHCGSTGTRVSSPSGTVAGSYFPGRDMGWVRITSADTVTPLVNRYNGGTVTVTGSQEAATGSSVCRSGATTGWRCGTIQSKNQTVRYAEGTVTGLTRTTACAEGGDSGGPWLTGSQAQGVTSGGTGDCRSGGITFFQPINPLLSYFGLQLVTG

SEQ ID NO: 4 - protein, 338 aa, Artificial Sequence
  Thermobifida fusca (F163Y_N267D)
MQELALKRDLGLSDAEVAELRAAEAEAVELEEELRDSLGSDFGGVYLDADTTEITVAVTDPAAVSRVDADDVTVDVVDFGETALNDFVASLNAIADTADPKVTGWYTDLESDAVVITTLRGGTPAAEELAERAGLDERAVRIVEEDEEPQSLAAIIGGNPYYYGNYRCSIGFSVRQGSQTGFATAGHCGSTGTRVSSPSGTVAGSYFPGRDMGWVRITSADTVTPLVNRYNGGTVTVTGSQEAATGSSVCRSGATTGWRCGTIQSKDQTVRYAEGTVTGLTRTTACAEGGDSGGPWLTGSQAQGVTSGGTGDCRSGGITFFQPINPLLSYFGLQLVTG

SEQ ID NO: 5 - protein, 338 aa, Artificial Sequence
  Thermobifida fusca (F163Y_N267S)
MQELALKRDLGLSDAEVAELRAAEAEAVELEEELRDSLGSDFGGVYLDADTTEITVAVTDPAAVSRVDADDVTVDVVDFGETALNDFVASLNAIADTADPKVTGWYTDLESDAVVITTLRGGTPAAEELAERAGLDERAVRIVEEDEEPQSLAAIIGGNPYYYGNYRCSIGFSVRQGSQTGFATAGHCGSTGTRVSSPSGTVAGSYFPGRDMGWVRITSADTVTPLVNRYNGGTVTVTGSQEAATGSSVCRSGATTGWRCGTIQSKSQTVRYAEGTVTGLTRTTACAEGGDSGGPWLTGSQAQGVTSGGTGDCRSGGITFFQPINPLLSYFGLQLVTG

SEQ ID NO: 6 - protein, 338 aa, Artificial Sequence
  Thermobifida fusca (F163S_N267D)
MQELALKRDLGLSDAEVAELRAAEAEAVELEEELRDSLGSDFGGVYLDADTTEITVAVTDPAAVSRVDADDVTVDVVDFGETALNDFVASLNAIADTADPKVTGWYTDLESDAVVITTLRGGTPAAEELAERAGLDERAVRIVEEDEEPQSLAAIIGGNPYYSGNYRCSIGFSVRQGSQTGFATAGHCGSTGTRVSSPSGTVAGSYFPGRDMGWVRITSADTVTPLVNRYNGGTVTVTGSQEAATGSSVCRSGATTGWRCGTIQSKDQTVRYAEGTVTGLTRTTACAEGGDSGGPWLTGSQAQGVTSGGTGDCRSGGITFFQPINPLLSYFGLQLVTG

SEQ ID NO: 7 - protein, 338 aa, Artificial Sequence
  Thermobifida fusca (F163S_N267T)
MQELALKRDLGLSDAEVAELRAAEAEAVELEEELRDSLGSDFGGVYLDADTTEITVAVTDPAAVSRVDADDVTVDVVDFGETALNDFVASLNAIADTADPKVTGWYTDLESDAVVITTLRGGTPAAEELAERAGLDERAVRIVEEDEEPQSLAAIIGGNPYYSGNYRCSIGFSVRQGSQTGFATAGHCGSTGTRVSSPSGTVAGSYFPGRDMGWVRITSADTVTPLVNRYNGGTVTVTGSQEAATGSSVCRSGATTGWRCGTIQSKTQTVRYAEGTVTGLTRTTACAEGGDSGGPWLTGSQAQGVTSGGTGDCRSGGITFFQPINPLLSYFGLQLVTG

SEQ ID NO: 8 - protein, 338 aa, Artificial Sequence
  Thermobifida fusca (F163A_N267G)
MQELALKRDLGLSDAEVAELRAAEAEAVELEEELRDSLGSDFGGVYLDADTTEITVAVTDPAAVSRVDADDVTVDVVDFGETALNDFVASLNAIADTADPKVTGWYTDLESDAVVITTLRGGTPAAEELAERAGLDERAVRIVEEDEEPQSLAAIIGGNPYYAGNYRCSIGFSVRQGSQTGFATAGHCGSTGTRVSSPSGTVAGSYFPGRDMGWVRITSADTVTPLVNRYNGGTVTVTGSQEAATGSSVCRSGATTGWRCGTIQSKGQTVRYAEGTVTGLTRTTACAEGGDSGGPWLTGSQAQGVTSGGTGDCRSGGITFFQPINPLLSYFGLQLVTG

SEQ ID NO: 9 - protein, 338 aa, Artificial Sequence
  Thermobifida fusca (F163A)
MQELALKRDLGLSDAEVAELRAAEAEAVELEEELRDSLGSDFGGVYLDADTTEITVAVTDPAAVSRVDADDVTVDVVDFGETALNDFVASLNAIADTADPKVTGWYTDLESDAVVITTLRGGTPAAEELAERAGLDERAVRIVEEDEEPQSLAAIIGGNPYYAGNYRCSIGFSVRQGSQTGFATAGHCGSTGTRVSSPSGTVAGSYFPGRDMGWVRITSADTVTPLVNRYNGGTVTVTGSQEAATGSSVCRSGATTGWRCGTIQSKNQTVRYAEGTVTGLTRTTACAEGGDSGGPWLTGSQAQGVTSGGTGDCRSGGITFFQPINPLLSYFGLQLVTG

SEQ ID NO: 10 - protein, 338 aa, Artificial Sequence
  Thermobifida fusca (F163R)
MQELALKRDLGLSDAEVAELRAAEAEAVELEEELRDSLGSDFGGVYLDADTTEITVAVTDPAAVSRVDADDVTVDVVDFGETALNDFVASLNAIADTADPKVTGWYTDLESDAVVITTLRGGTPAAEELAERAGLDERAVRIVEEDEEPQSLAAIIGGNPYYRGNYRCSIGFSVRQGSQTGFATAGHCGSTGTRVSSPSGTVAGSYFPGRDMGWVRITSADTVTPLVNRYNGGTVTVTGSQEAATGSSVCRSGATTGWRCGTIQSKNQTVRYAEGTVTGLTRTTACAEGGDSGGPWLTGSQAQGVTSGGTGDCRSGGITFFQPINPLLSYFGLQLVTG

SEQ ID NO: 11 - DNA, 47 bp, Artificial Sequence
  TAP_mature region_F
aagaagatgaagaaccacagagcttggctgcaattattggtggaaac

SEQ ID NO: 12 - DNA, 44 bp, Artificial Sequence
  TAP_mature region_R
gactgcaggtcgacaagctttcagccggtcactaattgaaggcc

SEQ ID NO: 13 - DNA, 23 bp, Artificial Sequence
  pBE-S-vector-F
aagcttgtcgacctgcagtctag

SEQ ID NO: 14 - DNA, 24 bp, Artificial Sequence
  pBE-S-vector-R
ctgtggttcttcatcttcttccac

SEQ ID NO: 15 - DNA, 37 bp, Artificial Sequence
  TAP_F12Y_F
gtggaaacccgtactattacggaaattacagatgcag

SEQ ID NO: 16 - DNA, 37 bp, Artificial Sequence
  TAP_F12Y_R
ctgcatctgtaatttccgtaatagtacgggtttccac

SEQ ID NO: 17 - DNA, 38 bp, Artificial Sequence
  TAP_N116D_F
ggaactatccaatcaaaagaccaaacggttcgctatgc

SEQ ID NO: 18 - DNA, 38 bp, Artificial Sequence
  TAP_N116D_R
gcatagcgaaccgtttggtcttttgattggatagttcc

SEQ ID NO: 19 - DNA, 37 bp, Artificial Sequence
  Saturation mutagenesis_F_1
gtggaaacccgtactatnnnggaaattacagatgcag

SEQ ID NO: 20 - DNA, 38 bp, Artificial Sequence
  Saturation mutagenesis_R_1
gcatagcgaaccgtttgnnnttttgattggatagttcc

SEQ ID NO: 21 - DNA, 38 bp, Artificial Sequence
  Saturation mutagenesis_F_2
ggaactatccaatcaaaannncaaacggttcgctatgc

SEQ ID NO: 22 - DNA, 37 bp, Artificial Sequence
  Saturation mutagenesis_R_2
ctgcatctgtaatttccnnnatagtacgggtttccac

SEQ ID NO: 23 - DNA, 1017 bp, Artificial Sequence
  Thermobifida fusca (F12Y)
atgcaagagctggcgttgaaacgggacctcggcctctctgacgcagaagtagccgaactccgggctgctgaggcggaagcggtcgagctcgaggaggagctccgcgattcattagggtcagacttcggcggtgtatatctggatgctgacaccaccgaaattacggtcgcggtaaccgacccggcagcggtaagtcgtgtcgacgcggatgatgtcacagttgatgttgtcgatttcggggaaacagctttgaatgattttgtggcttcattaaatgccattgccgacacggcagaccctaaagtcactggatggtataccgatctcgaaagtgatgccgtagtcattacgaccttgcgtggcgggactcctgctgccgaggaacttgctgagagagcgggtctcgacgaaagagccgttcggattgtggaagaagatgaagaaccacagagcttggctgcaattattggtggaaacccgtactattacggaaattacagatgcagtatcgggtttagtgtccgtcagggctctcaaacgggattcgcgaccgcaggccactgcggatccacggggacgcgtgtgtcttctccttcaggaacagttgcaggaagttatttcccgggtcgcgatatgggctgggtgcggattacatcagcagatactgtaacaccactcgtaaatcggtataatgggggaactgttacggtcactgggtcacaagaagctgccaccggatcctccgtttgtcgctctggagcaacaacgggctggcgctgcggaactatccaatcaaaaaaccaaacggttcgctatgcagaagggactgttactggtttaacaagaactacagcctgtgctgaaggtggggattctggagggccatggctcacaggtagccaggcgcaaggggttacaagcggcggaacaggcgattgcagaagtggagggattacctttttccaaccaatcaatccattgcttagctatttcggccttcaattagtgaccggctga

SEQ ID NO: 24 - DNA, 1017 bp, Artificial Sequence
  Thermobifida fusca (F163Y_N267D)
atgcaagagctggcgttgaaacgggacctcggcctctctgacgcagaagtagccgaactccgggctgctgaggcggaagcggtcgagctcgaggaggagctccgcgattcattagggtcagacttcggcggtgtatatctggatgctgacaccaccgaaattacggtcgcggtaaccgacccggcagcggtaagtcgtgtcgacgcggatgatgtcacagttgatgttgtcgatttcggggaaacagctttgaatgattttgtggcttcattaaatgccattgccgacacggcagaccctaaagtcactggatggtataccgatctcgaaagtgatgccgtagtcattacgaccttgcgtggcgggactcctgctgccgaggaacttgctgagagagcgggtctcgacgaaagagccgttcggattgtggaagaagatgaagaaccacagagcttggctgcaattattggtggaaacccgtactattacggaaattacagatgcagtatcgggtttagtgtccgtcagggctctcaaacgggattcgcgaccgcaggccactgcggatccacggggacgcgtgtgtcttctccttcaggaacagttgcaggaagttatttcccgggtcgcgatatgggctgggtgcggattacatcagcagatactgtaacaccactcgtaaatcggtataatgggggaactgttacggtcactgggtcacaagaagctgccaccggatcctccgtttgtcgctctggagcaacaacgggctggcgctgcggaactatccaatcaaaagaccaaacggttcgctatgcagaagggactgttactggtttaacaagaactacagcctgtgctgaaggtggggattctggagggccatggctcacaggtagccaggcgcaaggggttacaagcggcggaacaggcgattgcagaagtggagggattacctttttccaaccaatcaatccattgcttagctatttcggccttcaattagtgaccggctga

SEQ ID NO: 25 - DNA, 1017 bp, Artificial Sequence
  Thermobifida fusca (F163Y_N267S)
atgcaagagctggcgttgaaacgggacctcggcctctctgacgcagaagtagccgaactccgggctgctgaggcggaagcggtcgagctcgaggaggagctccgcgattcattagggtcagacttcggcggtgtatatctggatgctgacaccaccgaaattacggtcgcggtaaccgacccggcagcggtaagtcgtgtcgacgcggatgatgtcacagttgatgttgtcgatttcggggaaacagctttgaatgattttgtggcttcattaaatgccattgccgacacggcagaccctaaagtcactggatggtataccgatctcgaaagtgatgccgtagtcattacgaccttgcgtggcgggactcctgctgccgaggaacttgctgagagagcgggtctcgacgaaagagccgttcggattgtggaagaagatgaagaaccacagagcttggctgcaattattggtggaaacccgtactattacggaaattacagatgcagtatcgggtttagtgtccgtcagggctctcaaacgggattcgcgaccgcaggccactgcggatccacggggacgcgtgtgtcttctccttcaggaacagttgcaggaagttatttcccgggtcgcgatatgggctgggtgcggattacatcagcagatactgtaacaccactcgtaaatcggtataatgggggaactgttacggtcactgggtcacaagaagctgccaccggatcctccgtttgtcgctctggagcaacaacgggctggcgctgcggaactatccaatcaaaaagtcaaacggttcgctatgcagaagggactgttactggtttaacaagaactacagcctgtgctgaaggtggggattctggagggccatggctcacaggtagccaggcgcaaggggttacaagcggcggaacaggcgattgcagaagtggagggattacctttttccaaccaatcaatccattgcttagctatttcggccttcaattagtgaccggctga

SEQ ID NO: 26 - DNA, 1017 bp, Artificial Sequence
  Thermobifida fusca (F163S_N267D)
atgcaagagctggcgttgaaacgggacctcggcctctctgacgcagaagtagccgaactccgggctgctgaggcggaagcggtcgagctcgaggaggagctccgcgattcattagggtcagacttcggcggtgtatatctggatgctgacaccaccgaaattacggtcgcggtaaccgacccggcagcggtaagtcgtgtcgacgcggatgatgtcacagttgatgttgtcgatttcggggaaacagctttgaatgattttgtggcttcattaaatgccattgccgacacggcagaccctaaagtcactggatggtataccgatctcgaaagtgatgccgtagtcattacgaccttgcgtggcgggactcctgctgccgaggaacttgctgagagagcgggtctcgacgaaagagccgttcggattgtggaagaagatgaagaaccacagagcttggctgcaattattggtggaaacccgtactatagtggaaattacagatgcagtatcgggtttagtgtccgtcagggctctcaaacgggattcgcgaccgcaggccactgcggatccacggggacgcgtgtgtcttctccttcaggaacagttgcaggaagttatttcccgggtcgcgatatgggctgggtgcggattacatcagcagatactgtaacaccactcgtaaatcggtataatgggggaactgttacggtcactgggtcacaagaagctgccaccggatcctccgtttgtcgctctggagcaacaacgggctggcgctgcggaactatccaatcaaaagatcaaacggttcgctatgcagaagggactgttactggtttaacaagaactacagcctgtgctgaaggtggggattctggagggccatggctcacaggtagccaggcgcaaggggttacaagcggcggaacaggcgattgcagaagtggagggattacctttttccaaccaatcaatccattgcttagctatttcggccttcaattagtgaccggctga

SEQ ID NO: 27 - DNA, 1017 bp, Artificial Sequence
  Thermobifida fusca (F163S_N267T)
atgcaagagctggcgttgaaacgggacctcggcctctctgacgcagaagtagccgaactccgggctgctgaggcggaagcggtcgagctcgaggaggagctccgcgattcattagggtcagacttcggcggtgtatatctggatgctgacaccaccgaaattacggtcgcggtaaccgacccggcagcggtaagtcgtgtcgacgcggatgatgtcacagttgatgttgtcgatttcggggaaacagctttgaatgattttgtggcttcattaaatgccattgccgacacggcagaccctaaagtcactggatggtataccgatctcgaaagtgatgccgtagtcattacgaccttgcgtggcgggactcctgctgccgaggaacttgctgagagagcgggtctcgacgaaagagccgttcggattgtggaagaagatgaagaaccacagagcttggctgcaattattggtggaaacccgtactatagtggaaattacagatgcagtatcgggtttagtgtccgtcagggctctcaaacgggattcgcgaccgcaggccactgcggatccacggggacgcgtgtgtcttctccttcaggaacagttgcaggaagttatttcccgggtcgcgatatgggctgggtgcggattacatcagcagatactgtaacaccactcgtaaatcggtataatgggggaactgttacggtcactgggtcacaagaagctgccaccggatcctccgtttgtcgctctggagcaacaacgggctggcgctgcggaactatccaatcaaaaactcaaacggttcgctatgcagaagggactgttactggtttaacaagaactacagcctgtgctgaaggtggggattctggagggccatggctcacaggtagccaggcgcaaggggttacaagcggcggaacaggcgattgcagaagtggagggattacctttttccaaccaatcaatccattgcttagctatttcggccttcaattagtgaccggctga

SEQ ID NO: 28 - DNA, 1017 bp, Artificial Sequence
  Thermobifida fusca (F163A_N267G)
atgcaagagctggcgttgaaacgggacctcggcctctctgacgcagaagtagccgaactccgggctgctgaggcggaagcggtcgagctcgaggaggagctccgcgattcattagggtcagacttcggcggtgtatatctggatgctgacaccaccgaaattacggtcgcggtaaccgacccggcagcggtaagtcgtgtcgacgcggatgatgtcacagttgatgttgtcgatttcggggaaacagctttgaatgattttgtggcttcattaaatgccattgccgacacggcagaccctaaagtcactggatggtataccgatctcgaaagtgatgccgtagtcattacgaccttgcgtggcgggactcctgctgccgaggaacttgctgagagagcgggtctcgacgaaagagccgttcggattgtggaagaagatgaagaaccacagagcttggctgcaattattggtggaaacccgtactatgctggaaattacagatgcagtatcgggtttagtgtccgtcagggctctcaaacgggattcgcgaccgcaggccactgcggatccacggggacgcgtgtgtcttctccttcaggaacagttgcaggaagttatttcccgggtcgcgatatgggctgggtgcggattacatcagcagatactgtaacaccactcgtaaatcggtataatgggggaactgttacggtcactgggtcacaagaagctgccaccggatcctccgtttgtcgctctggagcaacaacgggctggcgctgcggaactatccaatcaaaaggtcaaacggttcgctatgcagaagggactgttactggtttaacaagaactacagcctgtgctgaaggtggggattctggagggccatggctcacaggtagccaggcgcaaggggttacaagcggcggaacaggcgattgcagaagtggagggattacctttttccaaccaatcaatccattgcttagctatttcggccttcaattagtgaccggctga

SEQ ID NO: 29 - DNA, 1017 bp, Artificial Sequence
  Thermobifida fusca (F163A)
atgcaagagctggcgttgaaacgggacctcggcctctctgacgcagaagtagccgaactccgggctgctgaggcggaagcggtcgagctcgaggaggagctccgcgattcattagggtcagacttcggcggtgtatatctggatgctgacaccaccgaaattacggtcgcggtaaccgacccggcagcggtaagtcgtgtcgacgcggatgatgtcacagttgatgttgtcgatttcggggaaacagctttgaatgattttgtggcttcattaaatgccattgccgacacggcagaccctaaagtcactggatggtataccgatctcgaaagtgatgccgtagtcattacgaccttgcgtggcgggactcctgctgccgaggaacttgctgagagagcgggtctcgacgaaagagccgttcggattgtggaagaagatgaagaaccacagagcttggctgcaattattggtggaaacccgtactatgctggaaattacagatgcagtatcgggtttagtgtccgtcagggctctcaaacgggattcgcgaccgcaggccactgcggatccacggggacgcgtgtgtcttctccttcaggaacagttgcaggaagttatttcccgggtcgcgatatgggctgggtgcggattacatcagcagatactgtaacaccactcgtaaatcggtataatgggggaactgttacggtcactgggtcacaagaagctgccaccggatcctccgtttgtcgctctggagcaacaacgggctggcgctgcggaactatccaatcaaaaaatcaaacggttcgctatgcagaagggactgttactggtttaacaagaactacagcctgtgctgaaggtggggattctggagggccatggctcacaggtagccaggcgcaaggggttacaagcggcggaacaggcgattgcagaagtggagggattacctttttccaaccaatcaatccattgcttagctatttcggccttcaattagtgaccggctga

SEQ ID NO: 30 - DNA, 1017 bp, Artificial Sequence
  Thermobifida fusca (F163R)
atgcaagagctggcgttgaaacgggacctcggcctctctgacgcagaagtagccgaactccgggctgctgaggcggaagcggtcgagctcgaggaggagctccgcgattcattagggtcagacttcggcggtgtatatctggatgctgacaccaccgaaattacggtcgcggtaaccgacccggcagcggtaagtcgtgtcgacgcggatgatgtcacagttgatgttgtcgatttcggggaaacagctttgaatgattttgtggcttcattaaatgccattgccgacacggcagaccctaaagtcactggatggtataccgatctcgaaagtgatgccgtagtcattacgaccttgcgtggcgggactcctgctgccgaggaacttgctgagagagcgggtctcgacgaaagagccgttcggattgtggaagaagatgaagaaccacagagcttggctgcaattattggtggaaacccgtactatagaggaaattacagatgcagtatcgggtttagtgtccgtcagggctctcaaacgggattcgcgaccgcaggccactgcggatccacggggacgcgtgtgtcttctccttcaggaacagttgcaggaagttatttcccgggtcgcgatatgggctgggtgcggattacatcagcagatactgtaacaccactcgtaaatcggtataatgggggaactgttacggtcactgggtcacaagaagctgccaccggatcctccgtttgtcgctctggagcaacaacgggctggcgctgcggaactatccaatcaaaaaatcaaacggttcgctatgcagaagggactgttactggtttaacaagaactacagcctgtgctgaaggtggggattctggagggccatggctcacaggtagccaggcgcaaggggttacaagcggcggaacaggcgattgcagaagtggagggattacctttttccaaccaatcaatccattgcttagctatttcggccttcaattagtgaccggctga

SEQ ID NO: 31 - protein, 187 aa, Unknown
  Thermobifida fusca_mature region
LAAIIGGNPYYFGNYRCSIGFSVRQGSQTGFATAGHCGSTGTRVSSPSGTVAGSYFPGRDMGWVRITSADTVTPLVNRYNGGTVTVTGSQEAATGSSVCRSGATTGWRCGTIQSKNQTVRYAEGTVTGLTRTTACAEGGDSGGPWLTGSQAQGVTSGGTGDCRSGGITFFQPINPLLSYFGLQLVTG

SEQ ID NO: 32 - protein, 187 aa, Artificial Sequence
  Thermobifida fusca_mature region (F12Y)
LAAIIGGNPYYYGNYRCSIGFSVRQGSQTGFATAGHCGSTGTRVSSPSGTVAGSYFPGRDMGWVRITSADTVTPLVNRYNGGTVTVTGSQEAATGSSVCRSGATTGWRCGTIQSKNQTVRYAEGTVTGLTRTTACAEGGDSGGPWLTGSQAQGVTSGGTGDCRSGGITFFQPINPLLSYFGLQLVTG

SEQ ID NO: 33 - protein, 187 aa, Artificial Sequence
  Thermobifida fusca_mature region (F12Y_N116D)
LAAIIGGNPYYYGNYRCSIGFSVRQGSQTGFATAGHCGSTGTRVSSPSGTVAGSYFPGRDMGWVRITSADTVTPLVNRYNGGTVTVTGSQEAATGSSVCRSGATTGWRCGTIQSKDQTVRYAEGTVTGLTRTTACAEGGDSGGPWLTGSQAQGVTSGGTGDCRSGGITFFQPINPLLSYFGLQLVTG

SEQ ID NO: 34 - protein, 187 aa, Artificial Sequence
  Thermobifida fusca_mature region (F12Y_N116S)
LAAIIGGNPYYYGNYRCSIGFSVRQGSQTGFATAGHCGSTGTRVSSPSGTVAGSYFPGRDMGWVRITSADTVTPLVNRYNGGTVTVTGSQEAATGSSVCRSGATTGWRCGTIQSKSQTVRYAEGTVTGLTRTTACAEGGDSGGPWLTGSQAQGVTSGGTGDCRSGGITFFQPINPLLSYFGLQLVTG

SEQ ID NO: 35 - protein, 187 aa, Artificial Sequence
  Thermobifida fusca_mature region (F12S_N116D)
LAAIIGGNPYYSGNYRCSIGFSVRQGSQTGFATAGHCGSTGTRVSSPSGTVAGSYFPGRDMGWVRITSADTVTPLVNRYNGGTVTVTGSQEAATGSSVCRSGATTGWRCGTIQSKDQTVRYAEGTVTGLTRTTACAEGGDSGGPWLTGSQAQGVTSGGTGDCRSGGITFFQPINPLLSYFGLQLVTG

SEQ ID NO: 36 - protein, 187 aa, Artificial Sequence
  Thermobifida fusca_mature region (F12S_N116T)
LAAIIGGNPYYSGNYRCSIGFSVRQGSQTGFATAGHCGSTGTRVSSPSGTVAGSYFPGRDMGWVRITSADTVTPLVNRYNGGTVTVTGSQEAATGSSVCRSGATTGWRCGTIQSKTQTVRYAEGTVTGLTRTTACAEGGDSGGPWLTGSQAQGVTSGGTGDCRSGGITFFQPINPLLSYFGLQLVTG

SEQ ID NO: 37 - protein, 187 aa, Artificial Sequence
  Thermobifida fusca_mature region (F12A_N116G)
LAAIIGGNPYYAGNYRCSIGFSVRQGSQTGFATAGHCGSTGTRVSSPSGTVAGSYFPGRDMGWVRITSADTVTPLVNRYNGGTVTVTGSQEAATGSSVCRSGATTGWRCGTIQSKGQTVRYAEGTVTGLTRTTACAEGGDSGGPWLTGSQAQGVTSGGTGDCRSGGITFFQPINPLLSYFGLQLVTG

SEQ ID NO: 38 - protein, 187 aa, Artificial Sequence
  Thermobifida fusca_mature region (F12A)
LAAIIGGNPYYAGNYRCSIGFSVRQGSQTGFATAGHCGSTGTRVSSPSGTVAGSYFPGRDMGWVRITSADTVTPLVNRYNGGTVTVTGSQEAATGSSVCRSGATTGWRCGTIQSKNQTVRYAEGTVTGLTRTTACAEGGDSGGPWLTGSQAQGVTSGGTGDCRSGGITFFQPINPLLSYFGLQLVTG

SEQ ID NO: 39 - protein, 187 aa, Artificial Sequence
  Thermobifida fusca_mature region (F12R)
LAAIIGGNPYYRGNYRCSIGFSVRQGSQTGFATAGHCGSTGTRVSSPSGTVAGSYFPGRDMGWVRITSADTVTPLVNRYNGGTVTVTGSQEAATGSSVCRSGATTGWRCGTIQSKNQTVRYAEGTVTGLTRTTACAEGGDSGGPWLTGSQAQGVTSGGTGDCRSGGITFFQPINPLLSYFGLQLVTG

SEQ ID NO: 40 - protein, 368 aa, Unknown
  Thermobifida fusca
MNHSSRRTTSLLFTAALAATALVAATTPASAQELALKRDLGLSDAEVAELRAAEAEAVELEEELRDSLGSDFGGVYLDADTTEITVAVTDPAAVSRVDADDVTVDVVDFGETALNDFVASLNAIADTADPKVTGWYTDLESDAVVITTLRGGTPAAEELAERAGLDERAVRIVEEDEEPQSLAAIIGGNPYYFGNYRCSIGFSVRQGSQTGFATAGHCGSTGTRVSSPSGTVAGSYFPGRDMGWVRITSADTVTPLVNRYNGGTVTVTGSQEAATGSSVCRSGATTGWRCGTIQSKNQTVRYAEGTVTGLTRTTACAEGGDSGGPWLTGSQAQGVTSGGTGDCRSGGITFFQPINPLLSYFGLQLVTG

SEQ ID NO: 41 - DNA, 564 bp, Artificial Sequence
  Thermobifida fusca_mature region (F12Y)
ttggctgcaattattggtggaaacccgtactattacggaaattacagatgcagtatcgggtttagtgtccgtcagggctctcaaacgggattcgcgaccgcaggccactgcggatccacggggacgcgtgtgtcttctccttcaggaacagttgcaggaagttatttcccgggtcgcgatatgggctgggtgcggattacatcagcagatactgtaacaccactcgtaaatcggtataatgggggaactgttacggtcactgggtcacaagaagctgccaccggatcctccgtttgtcgctctggagcaacaacgggctggcgctgcggaactatccaatcaaaaaaccaaacggttcgctatgcagaagggactgttactggtttaacaagaactacagcctgtgctgaaggtggggattctggagggccatggctcacaggtagccaggcgcaaggggttacaagcggcggaacaggcgattgcagaagtggagggattacctttttccaaccaatcaatccattgcttagctatttcggccttcaattagtgaccggctga

SEQ ID NO: 42 - DNA, 564 bp, Artificial Sequence
  Thermobifida fusca_mature region (F12Y_N116D)
ttggctgcaattattggtggaaacccgtactattacggaaattacagatgcagtatcgggtttagtgtccgtcagggctctcaaacgggattcgcgaccgcaggccactgcggatccacggggacgcgtgtgtcttctccttcaggaacagttgcaggaagttatttcccgggtcgcgatatgggctgggtgcggattacatcagcagatactgtaacaccactcgtaaatcggtataatgggggaactgttacggtcactgggtcacaagaagctgccaccggatcctccgtttgtcgctctggagcaacaacgggctggcgctgcggaactatccaatcaaaagaccaaacggttcgctatgcagaagggactgttactggtttaacaagaactacagcctgtgctgaaggtggggattctggagggccatggctcacaggtagccaggcgcaaggggttacaagcggcggaacaggcgattgcagaagtggagggattacctttttccaaccaatcaatccattgcttagctatttcggccttcaattagtgaccggctga

SEQ ID NO: 43 - DNA, 564 bp, Artificial Sequence
  Thermobifida fusca_mature region (F12Y_N116S)
ttggctgcaattattggtggaaacccgtactattacggaaattacagatgcagtatcgggtttagtgtccgtcagggctctcaaacgggattcgcgaccgcaggccactgcggatccacggggacgcgtgtgtcttctccttcaggaacagttgcaggaagttatttcccgggtcgcgatatgggctgggtgcggattacatcagcagatactgtaacaccactcgtaaatcggtataatgggggaactgttacggtcactgggtcacaagaagctgccaccggatcctccgtttgtcgctctggagcaacaacgggctggcgctgcggaactatccaatcaaaaagtcaaacggttcgctatgcagaagggactgttactggtttaacaagaactacagcctgtgctgaaggtggggattctggagggccatggctcacaggtagccaggcgcaaggggttacaagcggcggaacaggcgattgcagaagtggagggattacctttttccaaccaatcaatccattgcttagctatttcggccttcaattagtgaccggctga

SEQ ID NO: 44 - DNA, 564 bp, Artificial Sequence
  Thermobifida fusca_mature region (F12S_N116D)
ttggctgcaattattggtggaaacccgtactatagtggaaattacagatgcagtatcgggtttagtgtccgtcagggctctcaaacgggattcgcgaccgcaggccactgcggatccacggggacgcgtgtgtcttctccttcaggaacagttgcaggaagttatttcccgggtcgcgatatgggctgggtgcggattacatcagcagatactgtaacaccactcgtaaatcggtataatgggggaactgttacggtcactgggtcacaagaagctgccaccggatcctccgtttgtcgctctggagcaacaacgggctggcgctgcggaactatccaatcaaaagatcaaacggttcgctatgcagaagggactgttactggtttaacaagaactacagcctgtgctgaaggtggggattctggagggccatggctcacaggtagccaggcgcaaggggttacaagcggcggaacaggcgattgcagaagtggagggattacctttttccaaccaatcaatccattgcttagctatttcggccttcaattagtgaccggctga

SEQ ID NO: 45 - DNA, 564 bp, Artificial Sequence
  Thermobifida fusca_mature region (F12S_N116T)
ttggctgcaattattggtggaaacccgtactatagtggaaattacagatgcagtatcgggtttagtgtccgtcagggctctcaaacgggattcgcgaccgcaggccactgcggatccacggggacgcgtgtgtcttctccttcaggaacagttgcaggaagttatttcccgggtcgcgatatgggctgggtgcggattacatcagcagatactgtaacaccactcgtaaatcggtataatgggggaactgttacggtcactgggtcacaagaagctgccaccggatcctccgtttgtcgctctggagcaacaacgggctggcgctgcggaactatccaatcaaaaactcaaacggttcgctatgcagaagggactgttactggtttaacaagaactacagcctgtgctgaaggtggggattctggagggccatggctcacaggtagccaggcgcaaggggttacaagcggcggaacaggcgattgcagaagtggagggattacctttttccaaccaatcaatccattgcttagctatttcggccttcaattagtgaccggctga

SEQ ID NO: 46 - DNA, 564 bp, Artificial Sequence
  Thermobifida fusca_mature region (F12A_N116G)
ttggctgcaattattggtggaaacccgtactatgctggaaattacagatgcagtatcgggtttagtgtccgtcagggctctcaaacgggattcgcgaccgcaggccactgcggatccacggggacgcgtgtgtcttctccttcaggaacagttgcaggaagttatttcccgggtcgcgatatgggctgggtgcggattacatcagcagatactgtaacaccactcgtaaatcggtataatgggggaactgttacggtcactgggtcacaagaagctgccaccggatcctccgtttgtcgctctggagcaacaacgggctggcgctgcggaactatccaatcaaaaggtcaaacggttcgctatgcagaagggactgttactggtttaacaagaactacagcctgtgctgaaggtggggattctggagggccatggctcacaggtagccaggcgcaaggggttacaagcggcggaacaggcgattgcagaagtggagggattacctttttccaaccaatcaatccattgcttagctatttcggccttcaattagtgaccggctga

SEQ ID NO: 47 - DNA, 564 bp, Artificial Sequence
  Thermobifida fusca_mature region (F12A)
ttggctgcaattattggtggaaacccgtactatgctggaaattacagatgcagtatcgggtttagtgtccgtcagggctctcaaacgggattcgcgaccgcaggccactgcggatccacggggacgcgtgtgtcttctccttcaggaacagttgcaggaagttatttcccgggtcgcgatatgggctgggtgcggattacatcagcagatactgtaacaccactcgtaaatcggtataatgggggaactgttacggtcactgggtcacaagaagctgccaccggatcctccgtttgtcgctctggagcaacaacgggctggcgctgcggaactatccaatcaaaaaatcaaacggttcgctatgcagaagggactgttactggtttaacaagaactacagcctgtgctgaaggtggggattctggagggccatggctcacaggtagccaggcgcaaggggttacaagcggcggaacaggcgattgcagaagtggagggattacctttttccaaccaatcaatccattgcttagctatttcggccttcaattagtgaccggctga

SEQ ID NO: 48 - DNA, 564 bp, Artificial Sequence
  Thermobifida fusca_mature region (F12R)
ttggctgcaattattggtggaaacccgtactatagaggaaattacagatgcagtatcgggtttagtgtccgtcagggctctcaaacgggattcgcgaccgcaggccactgcggatccacggggacgcgtgtgtcttctccttcaggaacagttgcaggaagttatttcccgggtcgcgatatgggctgggtgcggattacatcagcagatactgtaacaccactcgtaaatcggtataatgggggaactgttacggtcactgggtcacaagaagctgccaccggatcctccgtttgtcgctctggagcaacaacgggctggcgctgcggaactatccaatcaaaaaatcaaacggttcgctatgcagaagggactgttactggtttaacaagaactacagcctgtgctgaaggtggggattctggagggccatggctcacaggtagccaggcgcaaggggttacaagcggcggaacaggcgattgcagaagtggagggattacctttttccaaccaatcaatccattgcttagctatttcggccttcaattagtgaccggctga